European Patent Application EP 4 631 967 A1, published October 15, 2025. Title: Peptide for cartilage regeneration and uses thereof. Applicant: CAREGEN CO., LTD. The sequence listing filed with the application follows.

SEQUENCE LISTING (16 sequences)

SEQ ID NO: 1 - protein, 13 aa, synthetic construct
SHIAGGLSFHSTV

SEQ ID NO: 2 - protein, 8 aa, synthetic construct
QSSLRALR

SEQ ID NO: 3 - DNA, 23 bp, synthetic construct
  source 1..23: mol_type = other DNA
ctatctggacgaagcagctggca

SEQ ID NO: 4 - DNA, 22 bp, synthetic construct
  source 1..22: mol_type = other DNA
atgggtgcaatgtcaatgatgg

SEQ ID NO: 5 - DNA, 20 bp, synthetic construct
  source 1..20: mol_type = other DNA
aactcagggcaggaggatgt

SEQ ID NO: 6 - DNA, 20 bp, synthetic construct
  source 1..20: mol_type = other DNA
tgtccttttggtcgtcgttc

SEQ ID NO: 7 - DNA, 20 bp, synthetic construct
  source 1..20: mol_type = other DNA
ccagcccgaacttgtaaaga

SEQ ID NO: 8 - DNA, 20 bp, synthetic construct
  source 1..20: mol_type = other DNA
tggacgcacaaccatcatac

SEQ ID NO: 9 - DNA, 20 bp, synthetic construct
  source 1..20: mol_type = other DNA
tgagtcctcaagcctcctgt

SEQ ID NO: 10 - DNA, 20 bp, synthetic construct
  source 1..20: mol_type = other DNA
gtgccagatcatcaccacac

SEQ ID NO: 11 - DNA, 20 bp, synthetic construct
  source 1..20: mol_type = other DNA
gcaggctatgagcagtgtga

SEQ ID NO: 12 - DNA, 20 bp, synthetic construct
  source 1..20: mol_type = other DNA
gcatacctcggaagcagaag

SEQ ID NO: 13 - DNA, 20 bp, synthetic construct
  source 1..20: mol_type = other DNA
accacagtccatgccatcac

SEQ ID NO: 14 - DNA, 20 bp, synthetic construct
  source 1..20: mol_type = other DNA
tccaccaccctgttgctgta

SEQ ID NO: 15 - DNA, 20 bp, synthetic construct
  source 1..20: mol_type = other DNA
gcggaggaagtcggtgaaga

SEQ ID NO: 16 - DNA, 20 bp, synthetic construct
  source 1..20: mol_type = other DNA
ccctctcgcttcaggtcagc